European Patent Specification EP 3 492 592 B1, published November 6, 2024. Title: Fibronectin fragment used for production of stem cell. Applicant: TAKARA BIO INC. The sequence listing filed with the application follows.

SEQUENCE LISTING (43 sequences)

SEQ ID NO: 1 - protein, 92 aa, Homo sapiens
SGPVEVFITETPSQPNSHPIQWNAPQPSHISKYILRWRPKNSVGRWKEATIPGHLNSYTIKGLKPGVVYEGQLISIQQYGHQEVTRFDFTTT

SEQ ID NO: 2 - protein, 91 aa, Homo sapiens
SPLVATSESVTEITASSFVVSWVSASDTVSGFRVEYELSEEGDEPQYLDLPSTATSVNIPDLLPGRKYIVNVYQISEDGEQSLILSTSQTT

SEQ ID NO: 3 - protein, 96 aa, Homo sapiens
APDAPPDPTVDQVDDTSIVVRWSRPQAPITGYRIVYSPSVEGSSTELNLPETANSVTLSDLQPGVQYNITIYAVEENQESTPVVIQQETTGTPRSD

SEQ ID NO: 4 - protein, 90 aa, Homo sapiens
TVPSPRDLQFVEVTDVKVTIMWTPPESAVTGYRVDVIPVNLPGEHGQRLPISRNTFAEVTGLSPGVTYYFKVFAVSHGRESKPLTAQQTT

SEQ ID NO: 5 - protein, 90 aa, Homo sapiens
KLDAPTNLQFVNETDSTVLVRWTPPRAQITGYRLTVGLTRRGQPRQYNVGPSVSKYPLRNLQPASEYTVSLVAIKGNQESPKATGVFTTL

SEQ ID NO: 6 - protein, 87 aa, Homo sapiens
QPGSSIPPYNTEVTETTIVITWTPAPRIGFKLGVRPSQGGEAPREVTSDSGSIVVSGLTPGVEYVYTIQVLRDGQERDAPIVNKVVT

SEQ ID NO: 7 - protein, 93 aa, Homo sapiens
PLSPPTNLHLEANPDTGVLTVSWERSTTPDITGYRITTTPTNGQQGNSLEEVVHADQSSCTFDNLSPGLEYNVSVYTVKDDKESVPISDTIIP

SEQ ID NO: 8 - protein, 87 aa, Homo sapiens
PTDLRFTNIGPDTMRVTWAPPPSIDLTNFLVRYSPVKNEEDVAELSISPSDNAVVLTNLLPGTEYVVSVSSVYEQHESTPLRGRQKT

SEQ ID NO: 9 - protein, 90 aa, Homo sapiens
GLDSPTGIDFSDITANSFTVHWIAPRATITGYRIRHHPEHFSGRPREDRVPHSRNSITLTNLTPGTEYVVSIVALNGREESPLLIGQQST

SEQ ID NO: 10 - protein, 94 aa, Homo sapiens
VSDVPRDLEVVAATPTSLLISWDAPAVTVRYYRITYGETGGNSPVQEFTVPGSKSTATISGLKPGVDYTITVYAVTGRGDSPASSKPISINYRT

SEQ ID NO: 11 - protein, 90 aa, Homo sapiens
EIDKPSQMQVTDVQDNSISVKWLPSSSPVTGYRVTTTPKNGPGPTKTKTAGPDQTEMTIEGLQPTVEYVVSVYAQNPSGESQPLVQTAVT

SEQ ID NO: 12 - protein, 92 aa, Homo sapiens
AIPAPTDLKFTQVTPTSLSAQWTPPNVQLTGYRVRVTPKEKTGPMKEINLAPDSSSVVVSGLMVATKYEVSVYALKDTLTSRPAQGVVTTLE

SEQ ID NO: 13 - protein, 89 aa, Homo sapiens
NVSPPRRARVTDATETTITISWRTKTETITGFQVDAVPANGQTPIQRTIKPDVRSYTITGLQPGTDYKIYLYTLNDNARSSPVVIDAST

SEQ ID NO: 14 - protein, 90 aa, Homo sapiens
AIDAPSNLRFLATTPNSLLVSWQPPRARITGYIIKYEKPGSPPREVVPRPRPGVTEATITGLEPGTEYTIYVIALKNNQKSEPLIGRKKT

SEQ ID NO: 15 - protein, 25 aa, Homo sapiens
DELPQLVTLPHPNLHGPEILDVPST

SEQ ID NO: 16 - protein, 932 aa, Artificial Sequence
  Fibronectin fragment named 120k-fr
SGPVEVFITETPSQPNSHPIQWNAPQPSHISKYILRWRPKNSVGRWKEATIPGHLNSYTIKGLKPGVVYEGQLISIQQYGHQEVTRFDFTTTSTSTPVTSNTVTGETTPFSPLVATSESVTEITASSFVVSWVSASDTVSGFRVEYELSEEGDEPQYLDLPSTATSVNIPDLLPGRKYIVNVYQISEDGEQSLILSTSQTTAPDAPPDPTVDQVDDTSIVVRWSRPQAPITGYRIVYSPSVEGSSTELNLPETANSVTLSDLQPGVQYNITIYAVEENQESTPVVIQQETTGTPRSDTVPSPRDLQFVEVTDVKVTIMWTPPESAVTGYRVDVIPVNLPGEHGQRLPISRNTFAEVTGLSPGVTYYFKVFAVSHGRESKPLTAQQTTKLDAPTNLQFVNETDSTVLVRWTPPRAQITGYRLTVGLTRRGQPRQYNVGPSVSKYPLRNLQPASEYTVSLVAIKGNQESPKATGVFTTLQPGSSIPPYNTEVTETTIVITWTPAPRIGFKLGVRPSQGGEAPREVTSDSGSIVVSGLTPGVEYVYTIQVLRDGQERDAPIVNKVVTPLSPPTNLHLEANPDTGVLTVSWERSTTPDITGYRITTTPTNGQQGNSLEEVVHADQSSCTFDNLSPGLEYNVSVYTVKDDKESVPISDTIIPAVPPPTDLRFTNIGPDTMRVTWAPPPSIDLTNFLVRYSPVKNEEDVAELSISPSDNAVVLTNLLPGTEYVVSVSSVYEQHESTPLRGRQKTGLDSPTGIDFSDITANSFTVHWIAPRATITGYRIRHHPEHFSGRPREDRVPHSRNSITLTNLTPGTEYVVSIVALNGREESPLLIGQQSTVSDVPRDLEVVAATPTSLLISWDAPAVTVRYYRITYGETGGNSPVQEFTVPGSKSTATISGLKPGVDYTITVYAVTGRGDSPASSKPISINYRT

SEQ ID NO: 17 - protein, 549 aa, Artificial Sequence
  Fibronectin fragment named CH-271
PTDLRFTNIGPDTMRVTWAPPPSIDLTNFLVRYSPVKNEEDVAELSISPSDNAVVLTNLLPGTEYVVSVSSVYEQHESTPLRGRQKTGLDSPTGIDFSDITANSFTVHWIAPRATITGYRIRHHPEHFSGRPREDRVPHSRNSITLTNLTPGTEYVVSIVALNGREESPLLIGQQSTVSDVPRDLEVVAATPTSLLISWDAPAVTVRYYRITYGETGGNSPVQEFTVPGSKSTATISGLKPGVDYTITVYAVTGRGDSPASSKPISINYRTEIDKPSMAIPAPTDLKFTQVTPTSLSAQWTPPNVQLTGYRVRVTPKEKTGPMKEINLAPDSSSVVVSGLMVATKYEVSVYALKDTLTSRPAQGVVTTLENVSPPRRARVTDATETTITISWRTKTETITGFQVDAVPANGQTPIQRTIKPDVRSYTITGLQPGTDYKIYLYTLNDNARSSPVVIDASTAIDAPSNLRFLATTPNSLLVSWQPPRARITGYIIKYEKPGSPPREVVPRPRPGVTEATITGLEPGTEYTIYVIALKNNQKSEPLIGRKKT

SEQ ID NO: 18 - protein, 574 aa, Artificial Sequence
  Fibronectin fragment named CH-296 (RetroNectin)
PTDLRFTNIGPDTMRVTWAPPPSIDLTNFLVRYSPVKNEEDVAELSISPSDNAVVLTNLLPGTEYVVSVSSVYEQHESTPLRGRQKTGLDSPTGIDFSDITANSFTVHWIAPRATITGYRIRHHPEHFSGRPREDRVPHSRNSITLTNLTPGTEYVVSIVALNGREESPLLIGQQSTVSDVPRDLEVVAATPTSLLISWDAPAVTVRYYRITYGETGGNSPVQEFTVPGSKSTATISGLKPGVDYTITVYAVTGRGDSPASSKPISINYRTEIDKPSMAIPAPTDLKFTQVTPTSLSAQWTPPNVQLTGYRVRVTPKEKTGPMKEINLAPDSSSVVVSGLMVATKYEVSVYALKDTLTSRPAQGVVTTLENVSPPRRARVTDATETTITISWRTKTETITGFQVDAVPANGQTPIQRTIKPDVRSYTITGLQPGTDYKIYLYTLNDNARSSPVVIDASTAIDAPSNLRFLATTPNSLLVSWQPPRARITGYIIKYEKPGSPPREVVPRPRPGVTEATITGLEPGTEYTIYVIALKNNQKSEPLIGRKKTDELPQLVTLPHPNLHGPEILDVPST

SEQ ID NO: 19 - protein, 881 aa, Artificial Sequence
  Fibronectin fragment named FCH-296
MSGPVEVFITETPSQPNSHPIQWNAPQPSHISKYILRWRPKNSVGRWKEATIPGHLNSYTIKGLKPGVVYEGQLISIQQYGHQEVTRFDFTTTSTSTPVTSNTVTGETTPFSPLVATSESVTEITASSFVVSWVSASDTVSGFRVEYELSEEGDEPQYLDLPSTATSVNIPDLLPGRKYIVNVYQISEDGEQSLILSTSQTTAPDAPPDPTVDQVDDTSIVVRWSRPQAPITGYRIVYSPSVEGSSTELNLPETANSVTLSDLQPGVQYNITIYAVEENQESTPVVIQQETTGTPRSDGSSGSSGSSPTDLRFTNIGPDTMRVTWAPPPSIDLTNFLVRYSPVKNEEDVAELSISPSDNAVVLTNLLPGTEYVVSVSSVYEQHESTPLRGRQKTGLDSPTGIDFSDITANSFTVHWIAPRATITGYRIRHHPEHFSGRPREDRVPHSRNSITLTNLTPGTEYVVSIVALNGREESPLLIGQQSTVSDVPRDLEVVAATPTSLLISWDAPAVTVRYYRITYGETGGNSPVQEFTVPGSKSTATISGLKPGVDYTITVYAVTGRGDSPASSKPISINYRTEIDKPSMAIPAPTDLKFTQVTPTSLSAQWTPPNVQLTGYRVRVTPKEKTGPMKEINLAPDSSSVVVSGLMVATKYEVSVYALKDTLTSRPAQGVVTTLENVSPPRRARVTDATETTITISWRTKTETITGFQVDAVPANGQTPIQRTIKPDVRSYTITGLQPGTDYKIYLYTLNDNARSSPVVIDASTAIDAPSNLRFLATTPNSLLVSWQPPRARITGYIIKYEKPGSPPREVVPRPRPGVTEATITGLEPGTEYTIYVIALKNNQKSEPLIGRKKTDELPQLVTLPHPNLHGPEILDVPST

SEQ ID NO: 20 - protein, 851 aa, Artificial Sequence
  Fibronectin fragment named DCH-296
MTVPSPRDLQFVEVTDVKVTIMWTPPESAVTGYRVDVIPVNLPGEHGQRLPISRNTFAEVTGLSPGVTYYFKVFAVSHGRESKPLTAQQTTKLDAPTNLQFVNETDSTVLVRWTPPRAQITGYRLTVGLTRRGQPRQYNVGPSVSKYPLRNLQPASEYTVSLVAIKGNQESPKATGVFTTLQPGSSIPPYNTEVTETTIVITWTPAPRIGFKLGVRPSQGGEAPREVTSDSGSIVVSGLTPGVEYVYTIQVLRDGQERDAPIVNKVVTGSSGSSGSSPTDLRFTNIGPDTMRVTWAPPPSIDLTNFLVRYSPVKNEEDVAELSISPSDNAVVLTNLLPGTEYVVSVSSVYEQHESTPLRGRQKTGLDSPTGIDFSDITANSFTVHWIAPRATITGYRIRHHPEHFSGRPREDRVPHSRNSITLTNLTPGTEYVVSIVALNGREESPLLIGQQSTVSDVPRDLEVVAATPTSLLISWDAPAVTVRYYRITYGETGGNSPVQEFTVPGSKSTATISGLKPGVDYTITVYAVTGRGDSPASSKPISINYRTEIDKPSMAIPAPTDLKFTQVTPTSLSAQWTPPNVQLTGYRVRVTPKEKTGPMKEINLAPDSSSVVVSGLMVATKYEVSVYALKDTLTSRPAQGVVTTLENVSPPRRARVTDATETTITISWRTKTETITGFQVDAVPANGQTPIQRTIKPDVRSYTITGLQPGTDYKIYLYTLNDNARSSPVVIDASTAIDAPSNLRFLATTPNSLLVSWQPPRARITGYIIKYEKPGSPPREVVPRPRPGVTEATITGLEPGTEYTIYVIALKNNQKSEPLIGRKKTDELPQLVTLPHPNLHGPEILDVPST

SEQ ID NO: 21 - protein, 887 aa, Artificial Sequence
  His-tag FCH-296
MHHHHHHSGPVEVFITETPSQPNSHPIQWNAPQPSHISKYILRWRPKNSVGRWKEATIPGHLNSYTIKGLKPGVVYEGQLISIQQYGHQEVTRFDFTTTSTSTPVTSNTVTGETTPFSPLVATSESVTEITASSFVVSWVSASDTVSGFRVEYELSEEGDEPQYLDLPSTATSVNIPDLLPGRKYIVNVYQISEDGEQSLILSTSQTTAPDAPPDPTVDQVDDTSIVVRWSRPQAPITGYRIVYSPSVEGSSTELNLPETANSVTLSDLQPGVQYNITIYAVEENQESTPVVIQQETTGTPRSDGSSGSSGSSPTDLRFTNIGPDTMRVTWAPPPSIDLTNFLVRYSPVKNEEDVAELSISPSDNAVVLTNLLPGTEYVVSVSSVYEQHESTPLRGRQKTGLDSPTGIDFSDITANSFTVHWIAPRATITGYRIRHHPEHFSGRPREDRVPHSRNSITLTNLTPGTEYVVSIVALNGREESPLLIGQQSTVSDVPRDLEVVAATPTSLLISWDAPAVTVRYYRITYGETGGNSPVQEFTVPGSKSTATISGLKPGVDYTITVYAVTGRGDSPASSKPISINYRTEIDKPSMAIPAPTDLKFTQVTPTSLSAQWTPPNVQLTGYRVRVTPKEKTGPMKEINLAPDSSSVVVSGLMVATKYEVSVYALKDTLTSRPAQGVVTTLENVSPPRRARVTDATETTITISWRTKTETITGFQVDAVPANGQTPIQRTIKPDVRSYTITGLQPGTDYKIYLYTLNDNARSSPVVIDASTAIDAPSNLRFLATTPNSLLVSWQPPRARITGYIIKYEKPGSPPREVVPRPRPGVTEATITGLEPGTEYTIYVIALKNNQKSEPLIGRKKTDELPQLVTLPHPNLHGPEILDVPST

SEQ ID NO: 22 - protein, 832 aa, Artificial Sequence
  His-tag DCH-296
MHHHHHHTVPSPRDLQFVEVTDVKVTIMWTPPESAVTGYRVDVIPVNLPGEHGQRLPISRNTFAEVTGLSPGVTYYFKVFAVSHGRESKPLTAQQTTKLDAPTNLQFVNETDSTVLVRWTPPRAQITGYRLTVGLTRRGQPRQYNVGPSVSKYPLRNLQPASEYTVSLVAIKGNQESPKATGVFTTLQPGSSIPPYNTEVTETTIVITWTPAPRIGFKLGVRPSQGGEAPREVTSDSGSIVVSGLTPGVEYVYTIQVLRDGQERDAPIVNKVVTGSSGSSGSSPTDLRFTNIGPDTMRVTWAPPPSIDLTNFLVRYSPVKNEEDVAELSISPSDNAVVLTNLLPGTEYVVSVSSVYEQHESTPLRGRQKTGLDSPTGIDFSDITANSFTVHWIAPRATITGYRIRHHPEHFSGRPREDRVPHSRNSITLTNLTPGTEYVVSIVALNGREESPLLIGQQSTVSDVPRDLEVVAATPTSLLISWDAPAVTVRYYRITYGETGGNSPVQEFTVPGSKSTATISGLKPGVDYTITVYAVTGRGDSPASSKPISINYRTEIDKPSMAIPAPTDLKFTQVTPTSLSAQWTPPNVQLTGYRVRVTPKEKTGPMKEINLAPDSSSVVVSGLMVATKYEVSVYALKDTLTSRPAQGVVTTLENVSPPRRARVTDATETTITISWRTKTETITGFQVDAVPANGQTPIQRTIKPDVRSYTITGLQPGTDYKIYLYTLNDNARSSPVVIDASTAIDAPSNLRFLATTPNSLLVSWQPPRARITGYIIKYEKPGSPPREVVPRPRPGVTEATITGLEPGTEYTIYVIALKNNQKSEPLIGRKKT

SEQ ID NO: 23 - protein, 83 aa, Artificial Sequence
  N-terminal 9a.a. deletion of III-1
ETPSQPNSHPIQWNAPQPSHISKYILRWRPKNSVGRWKEATIPGHLNSYTIKGLKPGVVYEGQLISIQQYGHQEVTRFDFTTT

SEQ ID NO: 24 - protein, 87 aa, Artificial Sequence
  N-terminal 5a.a. deletion of III-1
VFITETPSQPNSHPIQWNAPQPSHISKYILRWRPKNSVGRWKEATIPGHLNSYTIKGLKPGVVYEGQLISIQQYGHQEVTRFDFTTT

SEQ ID NO: 25 - protein, 89 aa, Artificial Sequence
  N-terminal 3a.a. deletion of III-1
VEVFITETPSQPNSHPIQWNAPQPSHISKYILRWRPKNSVGRWKEATIPGHLNSYTIKGLKPGVVYEGQLISIQQYGHQEVTRFDFTTT

SEQ ID NO: 26 - protein, 682 aa, Artificial Sequence
  His-tag F1CH-296
MHHHHHHSGPVEVFITETPSQPNSHPIQWNAPQPSHISKYILRWRPKNSVGRWKEATIPGHLNSYTIKGLKPGVVYEGQLISIQQYGHQEVTRFDFTTTGSSGSSGSSPTDLRFTNIGPDTMRVTWAPPPSIDLTNFLVRYSPVKNEEDVAELSISPSDNAVVLTNLLPGTEYVVSVSSVYEQHESTPLRGRQKTGLDSPTGIDFSDITANSFTVHWIAPRATITGYRIRHHPEHFSGRPREDRVPHSRNSITLTNLTPGTEYVVSIVALNGREESPLLIGQQSTVSDVPRDLEVVAATPTSLLISWDAPAVTVRYYRITYGETGGNSPVQEFTVPGSKSTATISGLKPGVDYTITVYAVTGRGDSPASSKPISINYRTEIDKPSMAIPAPTDLKFTQVTPTSLSAQWTPPNVQLTGYRVRVTPKEKTGPMKEINLAPDSSSVVVSGLMVATKYEVSVYALKDTLTSRPAQGVVTTLENVSPPRRARVTDATETTITISWRTKTETITGFQVDAVPANGQTPIQRTIKPDVRSYTITGLQPGTDYKIYLYTLNDNARSSPVVIDASTAIDAPSNLRFLATTPNSLLVSWQPPRARITGYIIKYEKPGSPPREVVPRPRPGVTEATITGLEPGTEYTIYVIALKNNQKSEPLIGRKKTDELPQLVTLPHPNLHGPEILDVPST

SEQ ID NO: 27 - protein, 699 aa, Artificial Sequence
  His-tag F2CH-296
MHHHHHHSTSTPVTSNTVTGETTPFSPLVATSESVTEITASSFVVSWVSASDTVSGFRVEYELSEEGDEPQYLDLPSTATSVNIPDLLPGRKYIVNVYQISEDGEQSLILSTSQTTGSSGSSGSSPTDLRFTNIGPDTMRVTWAPPPSIDLTNFLVRYSPVKNEEDVAELSISPSDNAVVLTNLLPGTEYVVSVSSVYEQHESTPLRGRQKTGLDSPTGIDFSDITANSFTVHWIAPRATITGYRIRHHPEHFSGRPREDRVPHSRNSITLTNLTPGTEYVVSIVALNGREESPLLIGQQSTVSDVPRDLEVVAATPTSLLISWDAPAVTVRYYRITYGETGGNSPVQEFTVPGSKSTATISGLKPGVDYTITVYAVTGRGDSPASSKPISINYRTEIDKPSMAIPAPTDLKFTQVTPTSLSAQWTPPNVQLTGYRVRVTPKEKTGPMKEINLAPDSSSVVVSGLMVATKYEVSVYALKDTLTSRPAQGVVTTLENVSPPRRARVTDATETTITISWRTKTETITGFQVDAVPANGQTPIQRTIKPDVRSYTITGLQPGTDYKIYLYTLNDNARSSPVVIDASTAIDAPSNLRFLATTPNSLLVSWQPPRARITGYIIKYEKPGSPPREVVPRPRPGVTEATITGLEPGTEYTIYVIALKNNQKSEPLIGRKKTDELPQLVTLPHPNLHGPEILDVPST

SEQ ID NO: 28 - protein, 686 aa, Artificial Sequence
  His-tag F3CH-296
MHHHHHHAPDAPPDPTVDQVDDTSIVVRWSRPQAPITGYRIVYSPSVEGSSTELNLPETANSVTLSDLQPGVQYNITIYAVEENQESTPVVIQQETTGTPRSDGSSGSSGSSPTDLRFTNIGPDTMRVTWAPPPSIDLTNFLVRYSPVKNEEDVAELSISPSDNAVVLTNLLPGTEYVVSVSSVYEQHESTPLRGRQKTGLDSPTGIDFSDITANSFTVHWIAPRATITGYRIRHHPEHFSGRPREDRVPHSRNSITLTNLTPGTEYVVSIVALNGREESPLLIGQQSTVSDVPRDLEVVAATPTSLLISWDAPAVTVRYYRITYGETGGNSPVQEFTVPGSKSTATISGLKPGVDYTITVYAVTGRGDSPASSKPISINYRTEIDKPSMAIPAPTDLKFTQVTPTSLSAQWTPPNVQLTGYRVRVTPKEKTGPMKEINLAPDSSSVVVSGLMVATKYEVSVYALKDTLTSRPAQGVVTTLENVSPPRRARVTDATETTITISWRTKTETITGFQVDAVPANGQTPIQRTIKPDVRSYTITGLQPGTDYKIYLYTLNDNARSSPVVIDASTAIDAPSNLRFLATTPNSLLVSWQPPRARITGYIIKYEKPGSPPREVVPRPRPGVTEATITGLEPGTEYTIYVIALKNNQKSEPLIGRKKTDELPQLVTLPHPNLHGPEILDVPST

SEQ ID NO: 29 - protein, 872 aa, Artificial Sequence
  N-terminal 9a.a. deletion of FCH-296
METPSQPNSHPIQWNAPQPSHISKYILRWRPKNSVGRWKEATIPGHLNSYTIKGLKPGVVYEGQLISIQQYGHQEVTRFDFTTTSTSTPVTSNTVTGETTPFSPLVATSESVTEITASSFVVSWVSASDTVSGFRVEYELSEEGDEPQYLDLPSTATSVNIPDLLPGRKYIVNVYQISEDGEQSLILSTSQTTAPDAPPDPTVDQVDDTSIVVRWSRPQAPITGYRIVYSPSVEGSSTELNLPETANSVTLSDLQPGVQYNITIYAVEENQESTPVVIQQETTGTPRSDGSSGSSGSSPTDLRFTNIGPDTMRVTWAPPPSIDLTNFLVRYSPVKNEEDVAELSISPSDNAVVLTNLLPGTEYVVSVSSVYEQHESTPLRGRQKTGLDSPTGIDFSDITANSFTVHWIAPRATITGYRIRHHPEHFSGRPREDRVPHSRNSITLTNLTPGTEYVVSIVALNGREESPLLIGQQSTVSDVPRDLEVVAATPTSLLISWDAPAVTVRYYRITYGETGGNSPVQEFTVPGSKSTATISGLKPGVDYTITVYAVTGRGDSPASSKPISINYRTEIDKPSMAIPAPTDLKFTQVTPTSLSAQWTPPNVQLTGYRVRVTPKEKTGPMKEINLAPDSSSVVVSGLMVATKYEVSVYALKDTLTSRPAQGVVTTLENVSPPRRARVTDATETTITISWRTKTETITGFQVDAVPANGQTPIQRTIKPDVRSYTITGLQPGTDYKIYLYTLNDNARSSPVVIDASTAIDAPSNLRFLATTPNSLLVSWQPPRARITGYIIKYEKPGSPPREVVPRPRPGVTEATITGLEPGTEYTIYVIALKNNQKSEPLIGRKKTDELPQLVTLPHPNLHGPEILDVPST

SEQ ID NO: 30 - protein, 875 aa, Artificial Sequence
  N-terminal 6a.a. deletion of FCH-296
MFITETPSQPNSHPIQWNAPQPSHISKYILRWRPKNSVGRWKEATIPGHLNSYTIKGLKPGVVYEGQLISIQQYGHQEVTRFDFTTTSTSTPVTSNTVTGETTPFSPLVATSESVTEITASSFVVSWVSASDTVSGFRVEYELSEEGDEPQYLDLPSTATSVNIPDLLPGRKYIVNVYQISEDGEQSLILSTSQTTAPDAPPDPTVDQVDDTSIVVRWSRPQAPITGYRIVYSPSVEGSSTELNLPETANSVTLSDLQPGVQYNITIYAVEENQESTPVVIQQETTGTPRSDGSSGSSGSSPTDLRFTNIGPDTMRVTWAPPPSIDLTNFLVRYSPVKNEEDVAELSISPSDNAVVLTNLLPGTEYVVSVSSVYEQHESTPLRGRQKTGLDSPTGIDFSDITANSFTVHWIAPRATITGYRIRHHPEHFSGRPREDRVPHSRNSITLTNLTPGTEYVVSIVALNGREESPLLIGQQSTVSDVPRDLEVVAATPTSLLISWDAPAVTVRYYRITYGETGGNSPVQEFTVPGSKSTATISGLKPGVDYTITVYAVTGRGDSPASSKPISINYRTEIDKPSMAIPAPTDLKFTQVTPTSLSAQWTPPNVQLTGYRVRVTPKEKTGPMKEINLAPDSSSVVVSGLMVATKYEVSVYALKDTLTSRPAQGVVTTLENVSPPRRARVTDATETTITISWRTKTETITGFQVDAVPANGQTPIQRTIKPDVRSYTITGLQPGTDYKIYLYTLNDNARSSPVVIDASTAIDAPSNLRFLATTPNSLLVSWQPPRARITGYIIKYEKPGSPPREVVPRPRPGVTEATITGLEPGTEYTIYVIALKNNQKSEPLIGRKKTDELPQLVTLPHPNLHGPEILDVPST

SEQ ID NO: 31 - protein, 876 aa, Artificial Sequence
  N-terminal 5a.a. deletion of FCH-296
MVFITETPSQPNSHPIQWNAPQPSHISKYILRWRPKNSVGRWKEATIPGHLNSYTIKGLKPGVVYEGQLISIQQYGHQEVTRFDFTTTSTSTPVTSNTVTGETTPFSPLVATSESVTEITASSFVVSWVSASDTVSGFRVEYELSEEGDEPQYLDLPSTATSVNIPDLLPGRKYIVNVYQISEDGEQSLILSTSQTTAPDAPPDPTVDQVDDTSIVVRWSRPQAPITGYRIVYSPSVEGSSTELNLPETANSVTLSDLQPGVQYNITIYAVEENQESTPVVIQQETTGTPRSDGSSGSSGSSPTDLRFTNIGPDTMRVTWAPPPSIDLTNFLVRYSPVKNEEDVAELSISPSDNAVVLTNLLPGTEYVVSVSSVYEQHESTPLRGRQKTGLDSPTGIDFSDITANSFTVHWIAPRATITGYRIRHHPEHFSGRPREDRVPHSRNSITLTNLTPGTEYVVSIVALNGREESPLLIGQQSTVSDVPRDLEVVAATPTSLLISWDAPAVTVRYYRITYGETGGNSPVQEFTVPGSKSTATISGLKPGVDYTITVYAVTGRGDSPASSKPISINYRTEIDKPSMAIPAPTDLKFTQVTPTSLSAQWTPPNVQLTGYRVRVTPKEKTGPMKEINLAPDSSSVVVSGLMVATKYEVSVYALKDTLTSRPAQGVVTTLENVSPPRRARVTDATETTITISWRTKTETITGFQVDAVPANGQTPIQRTIKPDVRSYTITGLQPGTDYKIYLYTLNDNARSSPVVIDASTAIDAPSNLRFLATTPNSLLVSWQPPRARITGYIIKYEKPGSPPREVVPRPRPGVTEATITGLEPGTEYTIYVIALKNNQKSEPLIGRKKTDELPQLVTLPHPNLHGPEILDVPST

SEQ ID NO: 32 - protein, 878 aa, Artificial Sequence
  N-terminal 3a.a. deletion of FCH-296
MVEVFITETPSQPNSHPIQWNAPQPSHISKYILRWRPKNSVGRWKEATIPGHLNSYTIKGLKPGVVYEGQLISIQQYGHQEVTRFDFTTTSTSTPVTSNTVTGETTPFSPLVATSESVTEITASSFVVSWVSASDTVSGFRVEYELSEEGDEPQYLDLPSTATSVNIPDLLPGRKYIVNVYQISEDGEQSLILSTSQTTAPDAPPDPTVDQVDDTSIVVRWSRPQAPITGYRIVYSPSVEGSSTELNLPETANSVTLSDLQPGVQYNITIYAVEENQESTPVVIQQETTGTPRSDGSSGSSGSSPTDLRFTNIGPDTMRVTWAPPPSIDLTNFLVRYSPVKNEEDVAELSISPSDNAVVLTNLLPGTEYVVSVSSVYEQHESTPLRGRQKTGLDSPTGIDFSDITANSFTVHWIAPRATITGYRIRHHPEHFSGRPREDRVPHSRNSITLTNLTPGTEYVVSIVALNGREESPLLIGQQSTVSDVPRDLEVVAATPTSLLISWDAPAVTVRYYRITYGETGGNSPVQEFTVPGSKSTATISGLKPGVDYTITVYAVTGRGDSPASSKPISINYRTEIDKPSMAIPAPTDLKFTQVTPTSLSAQWTPPNVQLTGYRVRVTPKEKTGPMKEINLAPDSSSVVVSGLMVATKYEVSVYALKDTLTSRPAQGVVTTLENVSPPRRARVTDATETTITISWRTKTETITGFQVDAVPANGQTPIQRTIKPDVRSYTITGLQPGTDYKIYLYTLNDNARSSPVVIDASTAIDAPSNLRFLATTPNSLLVSWQPPRARITGYIIKYEKPGSPPREVVPRPRPGVTEATITGLEPGTEYTIYVIALKNNQKSEPLIGRKKTDELPQLVTLPHPNLHGPEILDVPST

SEQ ID NO: 33 - protein, 884 aa, Artificial Sequence
  N-terminal 3a.a. insertion of FCH-296
MPSSSGPVEVFITETPSQPNSHPIQWNAPQPSHISKYILRWRPKNSVGRWKEATIPGHLNSYTIKGLKPGVVYEGQLISIQQYGHQEVTRFDFTTTSTSTPVTSNTVTGETTPFSPLVATSESVTEITASSFVVSWVSASDTVSGFRVEYELSEEGDEPQYLDLPSTATSVNIPDLLPGRKYIVNVYQISEDGEQSLILSTSQTTAPDAPPDPTVDQVDDTSIVVRWSRPQAPITGYRIVYSPSVEGSSTELNLPETANSVTLSDLQPGVQYNITIYAVEENQESTPVVIQQETTGTPRSDGSSGSSGSSPTDLRFTNIGPDTMRVTWAPPPSIDLTNFLVRYSPVKNEEDVAELSISPSDNAVVLTNLLPGTEYVVSVSSVYEQHESTPLRGRQKTGLDSPTGIDFSDITANSFTVHWIAPRATITGYRIRHHPEHFSGRPREDRVPHSRNSITLTNLTPGTEYVVSIVALNGREESPLLIGQQSTVSDVPRDLEVVAATPTSLLISWDAPAVTVRYYRITYGETGGNSPVQEFTVPGSKSTATISGLKPGVDYTITVYAVTGRGDSPASSKPISINYRTEIDKPSMAIPAPTDLKFTQVTPTSLSAQWTPPNVQLTGYRVRVTPKEKTGPMKEINLAPDSSSVVVSGLMVATKYEVSVYALKDTLTSRPAQGVVTTLENVSPPRRARVTDATETTITISWRTKTETITGFQVDAVPANGQTPIQRTIKPDVRSYTITGLQPGTDYKIYLYTLNDNARSSPVVIDASTAIDAPSNLRFLATTPNSLLVSWQPPRARITGYIIKYEKPGSPPREVVPRPRPGVTEATITGLEPGTEYTIYVIALKNNQKSEPLIGRKKTDELPQLVTLPHPNLHGPEILDVPST

SEQ ID NO: 34 - protein, 887 aa, Artificial Sequence
  N-terminal 6a.a. insertion of FCH-296
MQTYPSSSGPVEVFITETPSQPNSHPIQWNAPQPSHISKYILRWRPKNSVGRWKEATIPGHLNSYTIKGLKPGVVYEGQLISIQQYGHQEVTRFDFTTTSTSTPVTSNTVTGETTPFSPLVATSESVTEITASSFVVSWVSASDTVSGFRVEYELSEEGDEPQYLDLPSTATSVNIPDLLPGRKYIVNVYQISEDGEQSLILSTSQTTAPDAPPDPTVDQVDDTSIVVRWSRPQAPITGYRIVYSPSVEGSSTELNLPETANSVTLSDLQPGVQYNITIYAVEENQESTPVVIQQETTGTPRSDGSSGSSGSSPTDLRFTNIGPDTMRVTWAPPPSIDLTNFLVRYSPVKNEEDVAELSISPSDNAVVLTNLLPGTEYVVSVSSVYEQHESTPLRGRQKTGLDSPTGIDFSDITANSFTVHWIAPRATITGYRIRHHPEHFSGRPREDRVPHSRNSITLTNLTPGTEYVVSIVALNGREESPLLIGQQSTVSDVPRDLEVVAATPTSLLISWDAPAVTVRYYRITYGETGGNSPVQEFTVPGSKSTATISGLKPGVDYTITVYAVTGRGDSPASSKPISINYRTEIDKPSMAIPAPTDLKFTQVTPTSLSAQWTPPNVQLTGYRVRVTPKEKTGPMKEINLAPDSSSVVVSGLMVATKYEVSVYALKDTLTSRPAQGVVTTLENVSPPRRARVTDATETTITISWRTKTETITGFQVDAVPANGQTPIQRTIKPDVRSYTITGLQPGTDYKIYLYTLNDNARSSPVVIDASTAIDAPSNLRFLATTPNSLLVSWQPPRARITGYIIKYEKPGSPPREVVPRPRPGVTEATITGLEPGTEYTIYVIALKNNQKSEPLIGRKKTDELPQLVTLPHPNLHGPEILDVPST

SEQ ID NO: 35 - protein, 890 aa, Artificial Sequence
  N-terminal 9a.a. insertion of FCH-296
MQPLQTYPSSSGPVEVFITETPSQPNSHPIQWNAPQPSHISKYILRWRPKNSVGRWKEATIPGHLNSYTIKGLKPGVVYEGQLISIQQYGHQEVTRFDFTTTSTSTPVTSNTVTGETTPFSPLVATSESVTEITASSFVVSWVSASDTVSGFRVEYELSEEGDEPQYLDLPSTATSVNIPDLLPGRKYIVNVYQISEDGEQSLILSTSQTTAPDAPPDPTVDQVDDTSIVVRWSRPQAPITGYRIVYSPSVEGSSTELNLPETANSVTLSDLQPGVQYNITIYAVEENQESTPVVIQQETTGTPRSDGSSGSSGSSPTDLRFTNIGPDTMRVTWAPPPSIDLTNFLVRYSPVKNEEDVAELSISPSDNAVVLTNLLPGTEYVVSVSSVYEQHESTPLRGRQKTGLDSPTGIDFSDITANSFTVHWIAPRATITGYRIRHHPEHFSGRPREDRVPHSRNSITLTNLTPGTEYVVSIVALNGREESPLLIGQQSTVSDVPRDLEVVAATPTSLLISWDAPAVTVRYYRITYGETGGNSPVQEFTVPGSKSTATISGLKPGVDYTITVYAVTGRGDSPASSKPISINYRTEIDKPSMAIPAPTDLKFTQVTPTSLSAQWTPPNVQLTGYRVRVTPKEKTGPMKEINLAPDSSSVVVSGLMVATKYEVSVYALKDTLTSRPAQGVVTTLENVSPPRRARVTDATETTITISWRTKTETITGFQVDAVPANGQTPIQRTIKPDVRSYTITGLQPGTDYKIYLYTLNDNARSSPVVIDASTAIDAPSNLRFLATTPNSLLVSWQPPRARITGYIIKYEKPGSPPREVVPRPRPGVTEATITGLEPGTEYTIYVIALKNNQKSEPLIGRKKTDELPQLVTLPHPNLHGPEILDVPST

SEQ ID NO: 36 - protein, 892 aa, Artificial Sequence
  N-terminal 11a.a. insertion of FCH-296
MHCQPLQTYPSSSGPVEVFITETPSQPNSHPIQWNAPQPSHISKYILRWRPKNSVGRWKEATIPGHLNSYTIKGLKPGVVYEGQLISIQQYGHQEVTRFDFTTTSTSTPVTSNTVTGETTPFSPLVATSESVTEITASSFVVSWVSASDTVSGFRVEYELSEEGDEPQYLDLPSTATSVNIPDLLPGRKYIVNVYQISEDGEQSLILSTSQTTAPDAPPDPTVDQVDDTSIVVRWSRPQAPITGYRIVYSPSVEGSSTELNLPETANSVTLSDLQPGVQYNITIYAVEENQESTPVVIQQETTGTPRSDGSSGSSGSSPTDLRFTNIGPDTMRVTWAPPPSIDLTNFLVRYSPVKNEEDVAELSISPSDNAVVLTNLLPGTEYVVSVSSVYEQHESTPLRGRQKTGLDSPTGIDFSDITANSFTVHWIAPRATITGYRIRHHPEHFSGRPREDRVPHSRNSITLTNLTPGTEYVVSIVALNGREESPLLIGQQSTVSDVPRDLEVVAATPTSLLISWDAPAVTVRYYRITYGETGGNSPVQEFTVPGSKSTATISGLKPGVDYTITVYAVTGRGDSPASSKPISINYRTEIDKPSMAIPAPTDLKFTQVTPTSLSAQWTPPNVQLTGYRVRVTPKEKTGPMKEINLAPDSSSVVVSGLMVATKYEVSVYALKDTLTSRPAQGVVTTLENVSPPRRARVTDATETTITISWRTKTETITGFQVDAVPANGQTPIQRTIKPDVRSYTITGLQPGTDYKIYLYTLNDNARSSPVVIDASTAIDAPSNLRFLATTPNSLLVSWQPPRARITGYIIKYEKPGSPPREVVPRPRPGVTEATITGLEPGTEYTIYVIALKNNQKSEPLIGRKKTDELPQLVTLPHPNLHGPEILDVPST

SEQ ID NO: 37 - protein, 893 aa, Artificial Sequence
  N-terminal 12a.a. insertion of FCH-296
MWHCQPLQTYPSSSGPVEVFITETPSQPNSHPIQWNAPQPSHISKYILRWRPKNSVGRWKEATIPGHLNSYTIKGLKPGVVYEGQLISIQQYGHQEVTRFDFTTTSTSTPVTSNTVTGETTPFSPLVATSESVTEITASSFVVSWVSASDTVSGFRVEYELSEEGDEPQYLDLPSTATSVNIPDLLPGRKYIVNVYQISEDGEQSLILSTSQTTAPDAPPDPTVDQVDDTSIVVRWSRPQAPITGYRIVYSPSVEGSSTELNLPETANSVTLSDLQPGVQYNITIYAVEENQESTPVVIQQETTGTPRSDGSSGSSGSSPTDLRFTNIGPDTMRVTWAPPPSIDLTNFLVRYSPVKNEEDVAELSISPSDNAVVLTNLLPGTEYVVSVSSVYEQHESTPLRGRQKTGLDSPTGIDFSDITANSFTVHWIAPRATITGYRIRHHPEHFSGRPREDRVPHSRNSITLTNLTPGTEYVVSIVALNGREESPLLIGQQSTVSDVPRDLEVVAATPTSLLISWDAPAVTVRYYRITYGETGGNSPVQEFTVPGSKSTATISGLKPGVDYTITVYAVTGRGDSPASSKPISINYRTEIDKPSMAIPAPTDLKFTQVTPTSLSAQWTPPNVQLTGYRVRVTPKEKTGPMKEINLAPDSSSVVVSGLMVATKYEVSVYALKDTLTSRPAQGVVTTLENVSPPRRARVTDATETTITISWRTKTETITGFQVDAVPANGQTPIQRTIKPDVRSYTITGLQPGTDYKIYLYTLNDNARSSPVVIDASTAIDAPSNLRFLATTPNSLLVSWQPPRARITGYIIKYEKPGSPPREVVPRPRPGVTEATITGLEPGTEYTIYVIALKNNQKSEPLIGRKKTDELPQLVTLPHPNLHGPEILDVPST

SEQ ID NO: 38 - protein, 895 aa, Artificial Sequence
  N-terminal 14a.a. insertion of FCH-296
MGEWHCQPLQTYPSSSGPVEVFITETPSQPNSHPIQWNAPQPSHISKYILRWRPKNSVGRWKEATIPGHLNSYTIKGLKPGVVYEGQLISIQQYGHQEVTRFDFTTTSTSTPVTSNTVTGETTPFSPLVATSESVTEITASSFVVSWVSASDTVSGFRVEYELSEEGDEPQYLDLPSTATSVNIPDLLPGRKYIVNVYQISEDGEQSLILSTSQTTAPDAPPDPTVDQVDDTSIVVRWSRPQAPITGYRIVYSPSVEGSSTELNLPETANSVTLSDLQPGVQYNITIYAVEENQESTPVVIQQETTGTPRSDGSSGSSGSSPTDLRFTNIGPDTMRVTWAPPPSIDLTNFLVRYSPVKNEEDVAELSISPSDNAVVLTNLLPGTEYVVSVSSVYEQHESTPLRGRQKTGLDSPTGIDFSDITANSFTVHWIAPRATITGYRIRHHPEHFSGRPREDRVPHSRNSITLTNLTPGTEYVVSIVALNGREESPLLIGQQSTVSDVPRDLEVVAATPTSLLISWDAPAVTVRYYRITYGETGGNSPVQEFTVPGSKSTATISGLKPGVDYTITVYAVTGRGDSPASSKPISINYRTEIDKPSMAIPAPTDLKFTQVTPTSLSAQWTPPNVQLTGYRVRVTPKEKTGPMKEINLAPDSSSVVVSGLMVATKYEVSVYALKDTLTSRPAQGVVTTLENVSPPRRARVTDATETTITISWRTKTETITGFQVDAVPANGQTPIQRTIKPDVRSYTITGLQPGTDYKIYLYTLNDNARSSPVVIDASTAIDAPSNLRFLATTPNSLLVSWQPPRARITGYIIKYEKPGSPPREVVPRPRPGVTEATITGLEPGTEYTIYVIALKNNQKSEPLIGRKKTDELPQLVTLPHPNLHGPEILDVPST

SEQ ID NO: 39 - protein, 896 aa, Artificial Sequence
  N-terminal 15a.a. insertion of FCH-296
MIGEWHCQPLQTYPSSSGPVEVFITETPSQPNSHPIQWNAPQPSHISKYILRWRPKNSVGRWKEATIPGHLNSYTIKGLKPGVVYEGQLISIQQYGHQEVTRFDFTTTSTSTPVTSNTVTGETTPFSPLVATSESVTEITASSFVVSWVSASDTVSGFRVEYELSEEGDEPQYLDLPSTATSVNIPDLLPGRKYIVNVYQISEDGEQSLILSTSQTTAPDAPPDPTVDQVDDTSIVVRWSRPQAPITGYRIVYSPSVEGSSTELNLPETANSVTLSDLQPGVQYNITIYAVEENQESTPVVIQQETTGTPRSDGSSGSSGSSPTDLRFTNIGPDTMRVTWAPPPSIDLTNFLVRYSPVKNEEDVAELSISPSDNAVVLTNLLPGTEYVVSVSSVYEQHESTPLRGRQKTGLDSPTGIDFSDITANSFTVHWIAPRATITGYRIRHHPEHFSGRPREDRVPHSRNSITLTNLTPGTEYVVSIVALNGREESPLLIGQQSTVSDVPRDLEVVAATPTSLLISWDAPAVTVRYYRITYGETGGNSPVQEFTVPGSKSTATISGLKPGVDYTITVYAVTGRGDSPASSKPISINYRTEIDKPSMAIPAPTDLKFTQVTPTSLSAQWTPPNVQLTGYRVRVTPKEKTGPMKEINLAPDSSSVVVSGLMVATKYEVSVYALKDTLTSRPAQGVVTTLENVSPPRRARVTDATETTITISWRTKTETITGFQVDAVPANGQTPIQRTIKPDVRSYTITGLQPGTDYKIYLYTLNDNARSSPVVIDASTAIDAPSNLRFLATTPNSLLVSWQPPRARITGYIIKYEKPGSPPREVVPRPRPGVTEATITGLEPGTEYTIYVIALKNNQKSEPLIGRKKTDELPQLVTLPHPNLHGPEILDVPST

SEQ ID NO: 40 - protein, 889 aa, Artificial Sequence
  N-terminal HKRHEEGH insertion of FCH-296
MHKRHEEGHSGPVEVFITETPSQPNSHPIQWNAPQPSHISKYILRWRPKNSVGRWKEATIPGHLNSYTIKGLKPGVVYEGQLISIQQYGHQEVTRFDFTTTSTSTPVTSNTVTGETTPFSPLVATSESVTEITASSFVVSWVSASDTVSGFRVEYELSEEGDEPQYLDLPSTATSVNIPDLLPGRKYIVNVYQISEDGEQSLILSTSQTTAPDAPPDPTVDQVDDTSIVVRWSRPQAPITGYRIVYSPSVEGSSTELNLPETANSVTLSDLQPGVQYNITIYAVEENQESTPVVIQQETTGTPRSDGSSGSSGSSPTDLRFTNIGPDTMRVTWAPPPSIDLTNFLVRYSPVKNEEDVAELSISPSDNAVVLTNLLPGTEYVVSVSSVYEQHESTPLRGRQKTGLDSPTGIDFSDITANSFTVHWIAPRATITGYRIRHHPEHFSGRPREDRVPHSRNSITLTNLTPGTEYVVSIVALNGREESPLLIGQQSTVSDVPRDLEVVAATPTSLLISWDAPAVTVRYYRITYGETGGNSPVQEFTVPGSKSTATISGLKPGVDYTITVYAVTGRGDSPASSKPISINYRTEIDKPSMAIPAPTDLKFTQVTPTSLSAQWTPPNVQLTGYRVRVTPKEKTGPMKEINLAPDSSSVVVSGLMVATKYEVSVYALKDTLTSRPAQGVVTTLENVSPPRRARVTDATETTITISWRTKTETITGFQVDAVPANGQTPIQRTIKPDVRSYTITGLQPGTDYKIYLYTLNDNARSSPVVIDASTAIDAPSNLRFLATTPNSLLVSWQPPRARITGYIIKYEKPGSPPREVVPRPRPGVTEATITGLEPGTEYTIYVIALKNNQKSEPLIGRKKTDELPQLVTLPHPNLHGPEILDVPST

SEQ ID NO: 41 - protein, 885 aa, Artificial Sequence
  N-terminal HKRH insertion of FCH-296
MHKRHSGPVEVFITETPSQPNSHPIQWNAPQPSHISKYILRWRPKNSVGRWKEATIPGHLNSYTIKGLKPGVVYEGQLISIQQYGHQEVTRFDFTTTSTSTPVTSNTVTGETTPFSPLVATSESVTEITASSFVVSWVSASDTVSGFRVEYELSEEGDEPQYLDLPSTATSVNIPDLLPGRKYIVNVYQISEDGEQSLILSTSQTTAPDAPPDPTVDQVDDTSIVVRWSRPQAPITGYRIVYSPSVEGSSTELNLPETANSVTLSDLQPGVQYNITIYAVEENQESTPVVIQQETTGTPRSDGSSGSSGSSPTDLRFTNIGPDTMRVTWAPPPSIDLTNFLVRYSPVKNEEDVAELSISPSDNAVVLTNLLPGTEYVVSVSSVYEQHESTPLRGRQKTGLDSPTGIDFSDITANSFTVHWIAPRATITGYRIRHHPEHFSGRPREDRVPHSRNSITLTNLTPGTEYVVSIVALNGREESPLLIGQQSTVSDVPRDLEVVAATPTSLLISWDAPAVTVRYYRITYGETGGNSPVQEFTVPGSKSTATISGLKPGVDYTITVYAVTGRGDSPASSKPISINYRTEIDKPSMAIPAPTDLKFTQVTPTSLSAQWTPPNVQLTGYRVRVTPKEKTGPMKEINLAPDSSSVVVSGLMVATKYEVSVYALKDTLTSRPAQGVVTTLENVSPPRRARVTDATETTITISWRTKTETITGFQVDAVPANGQTPIQRTIKPDVRSYTITGLQPGTDYKIYLYTLNDNARSSPVVIDASTAIDAPSNLRFLATTPNSLLVSWQPPRARITGYIIKYEKPGSPPREVVPRPRPGVTEATITGLEPGTEYTIYVIALKNNQKSEPLIGRKKTDELPQLVTLPHPNLHGPEILDVPST

SEQ ID NO: 42 - protein, 883 aa, Artificial Sequence
  N-terminal HH insertion of FCH-296
MHHSGPVEVFITETPSQPNSHPIQWNAPQPSHISKYILRWRPKNSVGRWKEATIPGHLNSYTIKGLKPGVVYEGQLISIQQYGHQEVTRFDFTTTSTSTPVTSNTVTGETTPFSPLVATSESVTEITASSFVVSWVSASDTVSGFRVEYELSEEGDEPQYLDLPSTATSVNIPDLLPGRKYIVNVYQISEDGEQSLILSTSQTTAPDAPPDPTVDQVDDTSIVVRWSRPQAPITGYRIVYSPSVEGSSTELNLPETANSVTLSDLQPGVQYNITIYAVEENQESTPVVIQQETTGTPRSDGSSGSSGSSPTDLRFTNIGPDTMRVTWAPPPSIDLTNFLVRYSPVKNEEDVAELSISPSDNAVVLTNLLPGTEYVVSVSSVYEQHESTPLRGRQKTGLDSPTGIDFSDITANSFTVHWIAPRATITGYRIRHHPEHFSGRPREDRVPHSRNSITLTNLTPGTEYVVSIVALNGREESPLLIGQQSTVSDVPRDLEVVAATPTSLLISWDAPAVTVRYYRITYGETGGNSPVQEFTVPGSKSTATISGLKPGVDYTITVYAVTGRGDSPASSKPISINYRTEIDKPSMAIPAPTDLKFTQVTPTSLSAQWTPPNVQLTGYRVRVTPKEKTGPMKEINLAPDSSSVVVSGLMVATKYEVSVYALKDTLTSRPAQGVVTTLENVSPPRRARVTDATETTITISWRTKTETITGFQVDAVPANGQTPIQRTIKPDVRSYTITGLQPGTDYKIYLYTLNDNARSSPVVIDASTAIDAPSNLRFLATTPNSLLVSWQPPRARITGYIIKYEKPGSPPREVVPRPRPGVTEATITGLEPGTEYTIYVIALKNNQKSEPLIGRKKTDELPQLVTLPHPNLHGPEILDVPST

SEQ ID NO: 43 - protein, 884 aa, Artificial Sequence
  N-terminal HHH insertion of FCH-296
MHHHSGPVEVFITETPSQPNSHPIQWNAPQPSHISKYILRWRPKNSVGRWKEATIPGHLNSYTIKGLKPGVVYEGQLISIQQYGHQEVTRFDFTTTSTSTPVTSNTVTGETTPFSPLVATSESVTEITASSFVVSWVSASDTVSGFRVEYELSEEGDEPQYLDLPSTATSVNIPDLLPGRKYIVNVYQISEDGEQSLILSTSQTTAPDAPPDPTVDQVDDTSIVVRWSRPQAPITGYRIVYSPSVEGSSTELNLPETANSVTLSDLQPGVQYNITIYAVEENQESTPVVIQQETTGTPRSDGSSGSSGSSPTDLRFTNIGPDTMRVTWAPPPSIDLTNFLVRYSPVKNEEDVAELSISPSDNAVVLTNLLPGTEYVVSVSSVYEQHESTPLRGRQKTGLDSPTGIDFSDITANSFTVHWIAPRATITGYRIRHHPEHFSGRPREDRVPHSRNSITLTNLTPGTEYVVSIVALNGREESPLLIGQQSTVSDVPRDLEVVAATPTSLLISWDAPAVTVRYYRITYGETGGNSPVQEFTVPGSKSTATISGLKPGVDYTITVYAVTGRGDSPASSKPISINYRTEIDKPSMAIPAPTDLKFTQVTPTSLSAQWTPPNVQLTGYRVRVTPKEKTGPMKEINLAPDSSSVVVSGLMVATKYEVSVYALKDTLTSRPAQGVVTTLENVSPPRRARVTDATETTITISWRTKTETITGFQVDAVPANGQTPIQRTIKPDVRSYTITGLQPGTDYKIYLYTLNDNARSSPVVIDASTAIDAPSNLRFLATTPNSLLVSWQPPRARITGYIIKYEKPGSPPREVVPRPRPGVTEATITGLEPGTEYTIYVIALKNNQKSEPLIGRKKTDELPQLVTLPHPNLHGPEILDVPST